European Patent Specification EP 3 561 056 B1, published October 25, 2023. Title: Peptides for Treating Age-related Macular Degeneration. Applicant: DAIICHI SANKYO COMPANY, LIMITED. The sequence listing filed with the application follows.

SEQUENCE LISTING (56 sequences)

SEQ ID NO: 1 - protein, 63 aa, Homo sapiens
DPQFGLFSKYRTPNCSQYRLPGCPRHFNPVCGSDMSTYANECTLCMKIREGGHNIKIIRNGPC

SEQ ID NO: 2 - DNA, 192 bp, Homo sapiens
gatccgcagtttggtctgtttagcaaatatcgtaccccgaattgtagccagtatcgtctgcctggttgtccgcgtcattttaatccggtttgtggtagcgatatgagcacctatgcaaatgaatgtaccctgtgcatgaaaattcgtgaaggtggccataatattaaaattattcgcaatggtccgtgctaa

SEQ ID NO: 3 - protein, 65 aa, Artificial Sequence
  Artificial
DPQFGLFSKYRTPNCLKSEGMACYAYYEPVCGSDMSTYANECTLCMKIREGGHNIKIIRNGPCGG

SEQ ID NO: 4 - DNA, 198 bp, Artificial Sequence
  Artificial
gatccgcagtttggtctgtttagcaaatatcgtaccccgaattgtctgaaatctgaaggtatggcttgttacgcttactacgaaccggtttgtggtagcgatatgagcacctatgcaaatgaatgtaccctgtgcatgaaaattcgtgaaggtggccataatattaaaattattcgcaatggtccgtgcggcggctaa

SEQ ID NO: 5 - protein, 65 aa, Artificial Sequence
  Artificial
DPQFGLFSKYRTPNCTMDMGMACWAFYEPVCGSDMSTYANECTLCMKIREGGHNIKIIRNGPCGG

SEQ ID NO: 6 - DNA, 198 bp, Artificial Sequence
  Artificial
gatccgcagtttggtctgtttagcaaatatcgtaccccgaattgtactatggacatgggtatggcttgttgggctttctacgaaccggtttgtggtagcgatatgagcacctatgcaaatgaatgtaccctgtgcatgaaaattcgtgaaggtggccataatattaaaattattcgcaatggtccgtgcggcggctaa

SEQ ID NO: 7 - protein, 65 aa, Artificial Sequence
  Artificial
DPQFGLFSKYRTPNCGHYNGWACQAFFEPVCGSDMSTYANECTLCMKIREGGHNIKIIRNGPCGG

SEQ ID NO: 8 - DNA, 198 bp, Artificial Sequence
  Artificial
gatccgcagtttggtctgtttagcaaatatcgtaccccgaattgtggtcattacaacggttgggcttgtcaggctttcttcgaaccggtttgtggtagcgatatgagcacctatgcaaatgaatgtaccctgtgcatgaaaattcgtgaaggtggccataatattaaaattattcgcaatggtccgtgcggcggctaa

SEQ ID NO: 9 - protein, 65 aa, Artificial Sequence
  Artificial
DPQFGLFSKYRTPNCSDHAGMACVALYEPVCGSDMSTYENECVLCMKIREGGHNIKIIRNGPCGG

SEQ ID NO: 10 - DNA, 198 bp, Artificial Sequence
  Artificial
gatccgcagtttggtctgtttagcaaatatcgtaccccgaattgtagcgaccatgctggtatggcatgtgttgctctgtatgaaccggtttgtggtagcgatatgagcacctatgaaaatgaatgtgttctgtgcatgaaaattcgtgaaggtggccataatattaaaattattcgcaatggtccgtgcggcggctaa

SEQ ID NO: 11 - protein, 65 aa, Artificial Sequence
  Artificial
DPQFGLFSKYRTPNCSDFDGMACYAFYEPVCGSDMSTYMNECALCMKIREGGHNIKIIRNGPCGG

SEQ ID NO: 12 - DNA, 198 bp, Artificial Sequence
  Artificial
gatccgcagtttggtctgtttagcaaatatcgtaccccgaattgtagcgacttcgacggtatggcatgttacgctttctatgaaccggtttgtggtagcgatatgagcacctatatgaatgaatgtgctctgtgcatgaaaattcgtgaaggtggccataatattaaaattattcgcaatggtccgtgcggcggctaa

SEQ ID NO: 13 - protein, 65 aa, Artificial Sequence
  Artificial
DPQFGLFSKYRTPNCSQHEGMACYALYEPVCGSDMSTYVNECALCMKIREGGHNIKIIRNGPCGG

SEQ ID NO: 14 - DNA, 198 bp, Artificial Sequence
  Artificial
gatccgcagtttggtctgtttagcaaatatcgtaccccgaattgtagccagcatgaaggtatggcatgttacgctctgtatgaaccggtttgtggtagcgatatgagcacctatgttaatgaatgtgctctgtgcatgaaaattcgtgaaggtggccataatattaaaattattcgcaatggtccgtgcggcggctaa

SEQ ID NO: 15 - protein, 65 aa, Artificial Sequence
  Artificial
DPQFGLFSKYRTPNCSDHAGMACVALYEPVCGSDMSTYANECTLCMKIREGGHNIKIIRNGPCGG

SEQ ID NO: 16 - DNA, 198 bp, Artificial Sequence
  Artificial
gatccgcagtttggtctgtttagcaaatatcgtaccccgaattgtagcgaccatgctggtatggcatgtgttgctctgtatgaaccggtttgtggtagcgatatgagcacctatgcaaatgaatgtaccctgtgcatgaaaattcgtgaaggtggccataatattaaaattattcgcaatggtccgtgcggcggctaa

SEQ ID NO: 17 - protein, 65 aa, Artificial Sequence
  Artificial
DPQFGLFSKYRTPNCSDFDGMACYAFYEPVCGSDMSTYANECTLCMKIREGGHNIKIIRNGPCGG

SEQ ID NO: 18 - DNA, 198 bp, Artificial Sequence
  Artificial
gatccgcagtttggtctgtttagcaaatatcgtaccccgaattgtagcgacttcgacggtatggcatgttacgctttctatgaaccggtttgtggtagcgatatgagcacctatgcaaatgaatgtaccctgtgcatgaaaattcgtgaaggtggccataatattaaaattattcgcaatggtccgtgcggcggctaa

SEQ ID NO: 19 - protein, 65 aa, Artificial Sequence
  Artificial
DPQFGLFSKYRTPNCSQHEGMACYALYEPVCGSDMSTYANECTLCMKIREGGHNIKIIRNGPCGG

SEQ ID NO: 20 - DNA, 198 bp, Artificial Sequence
  Artificial
gatccgcagtttggtctgtttagcaaatatcgtaccccgaattgtagccagcatgaaggtatggcatgttacgctctgtatgaaccggtttgtggtagcgatatgagcacctatgcaaatgaatgtaccctgtgcatgaaaattcgtgaaggtggccataatattaaaattattcgcaatggtccgtgcggcggctaa

SEQ ID NO: 21 - protein, 65 aa, Artificial Sequence
  Artificial
DPQFGLFSKYRTPNCSDHAGMACVAFYEPVCGSDMSTYANECTLCMKIREGGHNIKIIRNGPCGG

SEQ ID NO: 22 - DNA, 198 bp, Artificial Sequence
  Artificial
gatccgcagtttggtctgtttagcaaatatcgtaccccgaattgtagcgaccatgctggtatggcatgtgttgctttttatgaaccggtttgtggtagcgatatgagcacctatgcaaatgaatgtaccctgtgcatgaaaattcgtgaaggtggccataatattaaaattattcgcaatggtccgtgcggcggctaa

SEQ ID NO: 23 - protein, 65 aa, Artificial Sequence
  Artificial
DPQFGLFSKYRTPNCADHAGMACVALYEPVCGSDMSTYENECVLCMKIREGGHNIKIIRNGPCGG

SEQ ID NO: 24 - protein, 65 aa, Artificial Sequence
  Artificial
GPQFGLFSKYRTPNCADHAGMACVALYEPVCGSDMSTYENECVLCMKIREGGHNIKIIRNGPCGG

SEQ ID NO: 25 - protein, 65 aa, Artificial Sequence
  Artificial
SPQFGLFSKYRTPNCADHAGMACVALYEPVCGSDMSTYENECVLCMKIREGGHNIKIIRNGPCGG

SEQ ID NO: 26 - protein, 65 aa, Artificial Sequence
  Artificial
EPQFGLFSKYRTPNCADHAGMACVALYEPVCGSDMSTYENECVLCMKIREGGHNIKIIRNGPCGG

SEQ ID NO: 27 - protein, 67 aa, Artificial Sequence
  Artificial
SLIPQFGLFSKYRTPNCADHAGMACVALYEPVCGSDMSTYENECVLCMKIREGGHNIKIIRNGPCGG

SEQ ID NO: 28 - protein, 65 aa, Artificial Sequence
  Artificial
GPQFGLFSKYRTPNCADFDGMACYAFYEPVCGSDMSTYANECTLCMKIREGGHNIKIIRNGPCGG

SEQ ID NO: 29 - protein, 65 aa, Artificial Sequence
  Artificial
GPQFGLFSKYRTPNCAQHEGMACYALYEPVCGSDMSTYANECTLCMKIREGGHNIKIIRNGPCGG

SEQ ID NO: 30 - protein, 63 aa, Artificial Sequence
  Artificial
  MISC_FEATURE (1)..(1): any amino acid
  MISC_FEATURE (16)..(19): any amino acid
  MISC_FEATURE (21)..(21): any amino acid
  MISC_FEATURE (24)..(24): any amino acid
  MISC_FEATURE (26)..(26): any amino acid
  MISC_FEATURE (27)..(27): any amino acid
  MISC_FEATURE (39)..(39): any amino acid
  MISC_FEATURE (43)..(43): any amino acid
XPQFGLFSKYRTPNCXXXXGXACXAXXEPVCGSDMSTYXNECXLCMKIREGGHNIKIIRNGPC

SEQ ID NO: 31 - protein, 39 aa, Artificial Sequence
  synthesized peptide
GSGMKETAAAKFERQHMDSPDLGTDDDDKAMADIGSANS

SEQ ID NO: 32 - protein, 6 aa, Artificial Sequence
  synthesized peptide
GASAAA

SEQ ID NO: 33 - DNA, 34 bp, Artificial Sequence
  primer
aaaagaattctgatccgcagtttggtctgtttag

SEQ ID NO: 34 - DNA, 40 bp, Artificial Sequence
  primer
aaaactcgagttatgcggccgcagacgcgccgcacggacc

SEQ ID NO: 35 - DNA, 45 bp, Artificial Sequence
  primer
aaaaggatccctggacaaacgtgatccgcagtttggtctgtttag

SEQ ID NO: 36 - DNA, 44 bp, Artificial Sequence
  primer
aaaactcgagttagccgccgcacggaccattgcgaataatttta

SEQ ID NO: 37 - DNA, 34 bp, Artificial Sequence
  primer
aaacatatggggcaggaagatcccaacagtttgc

SEQ ID NO: 38 - DNA, 33 bp, Artificial Sequence
  primer
aaactcgagtttggcctgtcggtcatgggactc

SEQ ID NO: 39 - DNA, 35 bp, Artificial Sequence
  primer
aaaagaattcgccaccatgcagattcctagagccg

SEQ ID NO: 40 - DNA, 36 bp, Artificial Sequence
  primer
aaaactcgagtcagtggtgatggtggtggtggccgg

SEQ ID NO: 41 - DNA, 42 bp, Artificial Sequence
  primer
cttgtcgtcatcgtccttgtagtcgccggggtcgatttcctc

SEQ ID NO: 42 - DNA, 44 bp, Artificial Sequence
  primer
gcgactacaaggacgatgacgacaagcaccaccaccatcatcac

SEQ ID NO: 43 - DNA, 41 bp, Artificial Sequence
  primer
aaaaactcgagctagtgatgatggtggtggtgcttgtcgtc

SEQ ID NO: 44 - DNA, 42 bp, Artificial Sequence
  primer
ccgcagtttggtctgtttagcaaatatcgtaccccgaattgt

SEQ ID NO: 45 - DNA, 43 bp, Artificial Sequence
  primer
gccataccagcatggtccgcacaattcggggtacgatatttgc

SEQ ID NO: 46 - DNA, 40 bp, Artifiicial Sequence
gcggaccatgctggtatggcatgtgttgctctgtatgaac

SEQ ID NO: 47 - DNA, 39 bp, Artificial Sequence
  primer
aaaactcgagttagccgccgcacggaccattgcgaataa

SEQ ID NO: 48 - DNA, 45 bp, Artificial Sequence; identical to SEQ ID NO: 35
  primer

SEQ ID NO: 49 - DNA, 45 bp, Artificial Sequence
  primer
aaaaggatccctggacaaacgtggcccgcagtttggtctgtttag

SEQ ID NO: 50 - DNA, 45 bp, artificial Sequence
  primer
aaaaggatccctggacaaacgtagcccgcagtttggtctgtttag

SEQ ID NO: 51 - DNA, 45 bp, Artificial Sequence
  primer
aaaaggatccctggacaaacgtgaaccgcagtttggtctgtttag

SEQ ID NO: 52 - DNA, 51 bp, Artificial Sequence
  primer
aaaaggatccctggacaaacgtagcctgattccgcagtttggtctgtttag

SEQ ID NO: 53 - protein, 458 aa, Homo sapiens
QLSRAGRSAPLAAGCPDRCEPARCPPQPEHCEGGRARDACGCCEVCGAPEGAACGLQEGPCGEGLQCVVPFGVPASATVRRRAQAGLCVCASSEPVCGSDANTYANLCQLRAASRRSERLHRPPVIVLQRGACGQGQEDPNSLRHKYNFIADVVEKIAPAVVHIELFRKLPFSKREVPVASGSGFIVSEDGLIVTNAHVVTNKHRVKVELKNGATYEAKIKDVDEKADIALIKIDHQGKLPVLLLGRSSELRPGEFVVAIGSPFSLQNTVTTGIVSTTQRGGKELGLRNSDMDYIQTDAIINYGNSGGPLVNLDGEVIGINTLKVTAGISFAIPSDKIKKFLTESHDRQAKGKAITKKKYIGIRMMSLTSSKAKELKDRHRDFPDVISGAYIIEVIPDTPAEAGGLKENDVIISINGQSVVSANDVSDVIKRESTLNMVVRRGNEDIMITVIPEEIDP

SEQ ID NO: 54 - protein, 10 aa, Artificial Sequence
  synthesized peptide
  BINDING (1)..(1): N-(4-methylcoumaryl-7-amide)-isoleucine
  BINDING (10)..(10): N epsilon-(2,4-dinitrophenyl)-lysine
XRRVSYSFKX

SEQ ID NO: 55 - DNA, 42 bp, Artificial Sequence
  primer
ccatcatcaactacggcaacgcgggcggacccctcgtgaacc

SEQ ID NO: 56 - DNA, 42 bp, Artificial Sequence
  primer
ggttcacgaggggtccgcccgcgttgccgtagttgatgatgg